European Patent Application EP 4 800 107 A1, published September 2, 2026. Title: 一种提升poly(A)质粒稳定性的宿主细胞. Applicant: 南京金斯瑞生物科技有限公司. Application CN. The sequence listing filed with the application follows.

SEQUENCE LISTING (50 sequences)

SEQ ID NO: 1 - DNA, 2628 bp, Escherichia coli
  source 1..2628: mol_type = genomic DNA
atgagcgaccttgcgagagaaattacaccggtcaacattgaggaagagctgaagagctcctatctggattatgcgatgtcggtcattgttggccgtgcgctgccagatgtccgagatggcctgaagccggtacaccgtcgcgtactttacgccatgaacgtactaggcaatgactggaacaaagcctataaaaaatctgcccgtgtcgttggtgacgtaatcggtaaataccatccccatggtgactcggcggtctatgacacgatcgtccgcatggcgcagccattctcgctgcgttatatgctggtagacggtcagggtaacttcggttctatcgacggcgactctgcggcggcaatgcgttatacggaaatccgtctggcgaaaattgcccatgaactgatggccgatctcgaaaaagagacggtcgatttcgttgataactatgacggcacggaaaaaattccggacgtcatgccaaccaaaattcctaacctgctggtgaacggttcttccggtatcgccgtaggtatggcaaccaacatcccgccgcacaacctgacggaagtcatcaacggttgtctggcgtatattgatgatgaagacatcagcattgaagggctgatggaacacatcccggggccggacttcccgacggcggcaatcattaacggtcgtcgcggtattgaagaagcttaccgtaccggtcgcggcaaggtgtatatccgcgctcgcgcagaagtggaagttgacgccaaaaccggtcgtgaaaccattatcgtccacgaaattccgtatcaggtaaacaaagcgcgcctgatcgagaagattgcggaactggtaaaagaaaaacgcgtggaaggcatcagcgcgctgcgtgacgagtctgacaaagacggtatgcgcatcgtgattgaagtgaaacgcgatgcggtcggtgaagttgtgctcaacaacctctactcccagacccagttgcaggtttctttcggtatcaacatggtggcattgcaccatggtcagccgaagatcatgaacctgaaagacatcatcgcggcgtttgttcgtcaccgccgtgaagtggtgacccgtcgtactattttcgaactgcgtaaagctcgcgatcgtgctcatatccttgaagcattagccgtggcgctggcgaacatcgacccgatcatcgaactgatccgtcatgcgccgacgcctgcagaagcgaaaactgcgctggttgctaatccgtggcagctgggcaacgttgccgcgatgctcgaacgtgctggcgacgatgctgcgcgtccggaatggctggagccagagttcggcgtgcgtgatggtctgtactacctgaccgaacagcaagctcaggcgattctggatctgcgtttgcagaaactgaccggtcttgagcacgaaaaactgctcgacgaatacaaagagctgctggatcagatcgcggaactgttgcgtattcttggtagcgccgatcgtctgatggaagtgatccgtgaagagctggagctggttcgtgaacagttcggtgacaaacgtcgtactgaaatcaccgccaacagcgcagacatcaacctggaagatctgatcacccaggaagatgtggtcgtgacgctctctcaccagggctacgttaagtatcagccgctttctgaatacgaagcgcagcgtcgtggcgggaaaggtaaatctgccgcacgtattaaagaagaagactttatcgaccgactgctggtggcgaacactcacgaccatattctgtgcttctccagccgtggtcgcgtctattcgatgaaagtttatcagttgccggaagccactcgtggcgcgcgcggtcgtccgatcgtcaacctgctgccgctggagcaggacgaacgtatcactgcgatcctgccagtgaccgagtttgaagaaggcgtgaaagtcttcatggcgaccgctaacggtaccgtgaagaaaactgtcctcaccgagttcaaccgtctgcgtaccgccggtaaagtggcgatcaaactggttgacggcgatgagctgatcggcgttgacctgaccagcggcgaagacgaagtaatgctgttctccgctgaaggtaaagtggtgcgctttaaagagtcttctgtccgtgcgatgggctgcaacaccaccggtgttcgcggtattcgcttaggtgaaggcgataaagtcgtctctctgatcgtgcctcgtggcgatggcgcaatcctcaccgcaacgcaaaacggttacggtaaacgtaccgcagtggcggaatacccaaccaagtcgcgtgcgacgaaaggggttatctccatcaaggttaccgaacgtaacggtttagttgttggcgcggtacaggtagatgactgcgaccagatcatgatgatcaccgatgccggtacgctggtacgtactcgcgtttcggaaatcagcatcgtgggccgtaacacccagggcgtgatcctcatccgtactgcggaagatgaaaacgtagtgggtctgcaacgtgttgctgaaccggttgacgaggaagatctggataccatcgacggcagtgccgcggaaggggacgatgaaatcgctccggaagtggacgttgacgacgagccagaagaagaataa

SEQ ID NO: 2 - DNA, 2415 bp, Escherichia coli
  source 1..2415: mol_type = genomic DNA
atgtcgaattcttatgactcctccagtatcaaagtcctgaaagggctggatgcggtgcgtaagcgcccgggtatgtatatcggcgacacggatgacggcaccggtctgcaccacatggtattcgaggtggtagataacgctatcgacgaagcgctcgcgggtcactgtaaagaaattatcgtcaccattcacgccgataactctgtctctgtacaggatgacgggcgcggcattccgaccggtattcacccggaagagggcgtatcggcggcggaagtgatcatgaccgttctgcacgcaggcggtaaatttgacgataactcctataaagtgtccggcggtctgcacggcgttggtgtttcggtagtaaacgccctgtcgcaaaaactggagctggttatccagcgcgagggtaaaattcaccgtcagatctacgaacacggtgtaccgcaggccccgctggcggttaccggcgagactgaaaaaaccggcaccatggtgcgtttctggcccagcctcgaaaccttcaccaatgtgaccgagttcgaatatgaaattctggcgaaacgtctgcgtgagttgtcgttcctcaactccggcgtttccattcgtctgcgcgacaagcgcgacggcaaagaagaccacttccactatgaaggcggcatcaaggcgttcgttgaatatctgaacaagaacaaaacgccgatccacccgaatatcttctacttctccactgaaaaagacggtattggcgtcgaagtggcgttgcagtggaacgatggcttccaggaaaacatctactgctttaccaacaacattccgcagcgtgacggcggtactcacctggcaggcttccgtgcggcgatgacccgtaccctgaacgcctacatggacaaagaaggctacagcaaaaaagccaaagtcagcgccaccggtgacgatgcgcgtgaaggcctgattgcggtcgtttccgtgaaagtgccggacccgaaattctcctcccagaccaaagacaaactggtttcttctgaggtgaaatcggcggttgaacagcagatgaacgaactgctggcagaatacctgctggaaaacccaaccgacgcgaaaatcgtggttggcaaaattatcgatgctgcccgtgcccgtgaagcggcgcgtcgcgcgcgtgaaatgacccgccgtaaaggtgcgctcgacttagcgggcctgccgggcaaactggcagactgccaggaacgcgatccggcgctttccgaactgtacctggtggaaggggactccgcgggcggctctgcgaagcaggggcgtaaccgcaagaaccaggcgattctgccgctgaagggtaaaatcctcaacgtcgagaaagcgcgcttcgataagatgctctcttctcaggaagtggcgacgcttatcaccgcgcttggctgtggtatcggtcgtgacgagtacaacccggacaaactgcgttatcacagcatcatcatcatgaccgatgcggacgtcgacggctcgcacattcgtacgctgctgttgaccttcttctatcgtcagatgccggaaatcgttgaacgcggtcacgtctacatcgctcagccgccgctgtacaaagtgaagaaaggcaagcaggaacagtacattaaagacgacgaagcgatggatcagtaccagatctctatcgcgctggacggcgcaacgctgcacaccaacgccagtgcaccggcattggctggcgaagcgttagagaaactggtatctgagtacaacgcgacgcagaaaatgatcaatcgtatggagcgtcgttatccgaaagcaatgctgaaagagcttatctatcagccgacgttgacggaagctgacctttctgatgagcagaccgttacccgctgggtgaacgcgctggtcagcgaactgaacgacaaagaacagcacggcagccagtggaagtttgatgttcacaccaatgctgagcaaaacctgttcgagccgattgttcgcgtgcgtacccacggtgtggatactgactatccgctggatcacgagtttatcaccggtggcgaatatcgtcgtatctgcacgctgggtgagaaactgcgtggcttgctggaagaagatgcgtttatcgaacgtggcgagcgtcgtcagccggtagccagcttcgagcaggcgctggactggctggtgaaagagtcccgtcgcggcctctccatccagcgttataaaggtctgggcgagatgaacccggaacagctgtgggaaaccactatggacccggaaagtcgtcgtatgctgcgcgttaccgttaaagatgcgattgctgccgaccagttgttcaccacgctgatgggcgacgccgttgaaccgcgccgtgcgtttattgaagagaacgccctgaaagcggcgaatatcgatatttaa

SEQ ID NO: 3 - DNA, 2628 bp, synthetic construct
  source 1..2628: mol_type = other DNA
atgagcgaccttgcgagagaaattacaccggtcaacattgaggaagagctgaagagctcctatctggattatgcgatgtctgtcattgttggccgtgcgctgccagatgtccgagatggcctgaagccggtacaccgtcgcgtactttacgccatgaacgtactaggcaatgactggaacaaagcctataaaaaatctgcccgtgtcgttggtgacgtaatcggtaaataccatcccgcaggtgactcggcggtctatgacacgatcgtccgcatggcgcagccattctcgctgcgttatatgctggtagacggtcagggtaacttcggttctatcgacggcgactctgcggcggcaatgcgttatacggaaatccgtctggcgaaaattgcccatgaactgatggccgatctcgaaaaagagacggtcgatttcgttgataactatgacggcacggaaaaaattccggacgtcatgccaaccaaaattcctaacctgctggtgaacggttcttccggtatcgccgtaggtatggcaaccaacatcccgccgcacaacctgacggaagtcatcaacggttgtctggcgtatattgatgatgaagacatcagcattgaagggctgatggaacacatcccggggccggacttcccgacggcggcaatcattaacggtcgtcgcggtattgaagaagcttaccgtaccggtcgcggcaaggtgtatatccgcgctcgcgcagaagtggaagttgacgccaaaaccggtcgtgaaaccattatcgtccacgaaattccgtatcaggtaaacaaagcgcgcctgatcgagaagattgcggaactggtaaaagaaaaacgcgtggaaggcatcagcgcgctgcgtgacgagtctgacaaagacggtatgcgcatcgtgattgaagtgaaacgcgatgcggtcggtgaagttgtgctcaacaacctctactcccagacccagttgcaggtttctttcggtatcaacatggtggcattgcaccatggtcagccgaagatcatgaacctgaaagacatcatcgcggcgtttgttcgtcaccgccgtgaagtggtgacccgtcgtactattttcgaactgcgtaaagctcgcgatcgtgctcatatccttgaagcattagccgtggcgctggcgaacatcgacccgatcatcgaactgatccgtcatgcgccgacgcctgcagaagcgaaaactgcgctggttgctaatccgtggcagctgggcaacgttgccgcgatgctcgaacgtgctggcgacgatgctgcgcgtccggaatggctggagccagagttcggcgtgcgtgatggtctgtactacctgaccgaacagcaagctcaggcgattctggatctgcgtttgcagaaactgaccggtcttgagcacgaaaaactgctcgacgaatacaaagagctgctggatcagatcgcggaactgttgcgtattcttggtagcgccgatcgtctgatggaagtgatccgtgaagagctggagctggttcgtgaacagttcggtgacaaacgtcgtactgaaatcaccgccaacagcgcagacatcaacctggaagatctgatcacccaggaagatgtggtcgtgacgctctctcaccagggctacgttaagtatcagccgctttctgaatacgaagcgcagcgtcgtggcgggaaaggtaaatctgccgcacgtattaaagaagaagactttatcgaccgactgctggtggcgaacactcacgaccatattctgtgcttctccagccgtggtcgcgtctattcgatgaaagtttatcagttgccggaagccactcgtggcgcgcgcggtcgtccgatcgtcaacctgctgccgctggagcaggacgaacgtatcactgcgatcctgccagtgaccgagtttgaagaaggcgtgaaagtcttcatggcgaccgctaacggtaccgtgaagaaaactgtcctcaccgagttcaaccgtctgcgtaccgccggtaaagtggcgatcaaactggttgacggcgatgagctgatcggcgttgacctgaccagcggcgaagacgaagtaatgctgttctccgctgaaggtaaagtggtgcgctttaaagagtcttctgtccgtgcgatgggctgcaacaccaccggtgttcgcggtattcgcttaggtgaaggcgataaagtcgtctctctgatcgtgcctcgtggcgatggcgcaatcctcaccgcaacgcaaaacggttacggtaaacgtaccgcagtggcggaatacccaaccaagtcgcgtgcgacgaaaggggttatctccatcaaggttaccgaacgtaacggtttagttgttggcgcggtacaggtagatgactgcgaccagatcatgatgatcaccgatgccggtacgctggtacgtactcgcgtttcggaaatcagcatcgtgggccgtaacacccagggcgtgatcctcatccgtactgcggaagatgaaaacgtagtgggtctgcaacgtgttgctgaaccggttgacgaggaagatctggataccatcgacggcagtgccgcggaaggggacgatgaaatcgctccggaagtggacgttgacgacgagccagaagaagaataa

SEQ ID NO: 4 - DNA, 2628 bp, synthetic construct
  source 1..2628: mol_type = other DNA
atgagcgaccttgcgagagaaattacaccggtcaacattgaggaagagctgaagagctcctatctggattatgcgatgtcggtcattgttggccgtgcgctgccagatgtccgagatggcctgaagccggtacaccgtcgcgtactttacgccatgaacgtactaggcaatgactggaacaaagcctataaaaaatctgcccgtgtcgttggtgacgtaatcggtaaataccatccccatggtgactcggcggtctatgacacgatcgtccgcatggcgcagccattctcgctgcgttatatgctggtagacggtcagggtaacttcggttctatcgacggcgactctgcggcggcaatgcgttatacggaaatccgtctggcgaaaattgcccatgaactgatggccgatctcgaaaaagagacggtcgatttcgttgataactatgacggcacggaaaaaattccggacgtcatgccaaccaaaattcctaacctgctggtgaacggttcttccggtatcgccgtaggtatggcaaccaacatcccgccgcacaacctgacggaagtcatcaacggttgtctggcgtatattgatgatgaagacatcagcattgaagggctgatggaacacatcccggggccggacttcccgacggcggcaatcattaacggtcgtcgcggtattgaagaagcttaccgtaccggtcgcggcaaggtgtatatccgcgctcgcgcagaagtggaagttgacgccaaaaccggtcgtgaaaccattatcgtccacgaaattccgtatcaggtaaacaaagcgcgcctgatcgagaagattgcggaactggtaaaagaaaaacgcgtggaaggcatcagcgcgctgcgtgacgagtctgacaaagacggtatgcgcatcgtgattgaagtgaaacgcgatgcggtcggtgaagttgtgctcaacaacctctactcccagacccagttgcaggtttctttcggtatcaacatggtggcattgcaccatggtcagccgaagatcatgaacctgaaagacatcatcgcggcgtttgttcgtcaccgccgtgaagtggtgacccgtcgtactattttcgaactgcgtaaagctcgcgatcgtgctcatatccttgaagcattagccgtggcgctggcgaacatcgacccgatcatcgaactgatccgtcatgcgccgacgcctgcagaagcgaaaactgcgctggttgctaatccgtggcagctgggcaacgttgccgcgatgctcgaacgtgctggcgacgatgctgcgcgtccggaatggctggagccagagttcggcgtgcgtgatggtctgtactacctgaccgaacagcaagctcaggcgattctggatctgcgtttgcagaaactgaccggtcttgagcacgaaaaactgctcgacgaatacaaagagctgctggatcagatcgcggaactgttgcgtattcttggtagcgccgatcgtctgatggaagtgatccgtgaagagctggagctggttcgtgaacagttcggtgacaaacgtcgtactgaaatcaccgccaacagcgcagacatcaacctcgaagatctgatcacccaggaagatgtggtcgtgacgctctctcaccagggctacgttaagtatcagccgctttctgaatacgaagcgcagcgtcgtggcgggaaaggtaaatctactgcacgtattaaagaagaagactttatcgaccgactgctggtggcgaacgcccacgaccatattctgtgcttctccagccgtggtcgcgtctattcgatgaaagtttatcagttgccggaagccactcgtggcgcgcgcggtcgtccgatcgtcaacctgctgccgctggagcaggacgaacgtatcactgcgatcctgccagtgaccgagtttgaagaaggcgtgaaagtcttcatggcgaccgctaacggtaccgtgaagaaaactgtcctcaccgagttcaaccgtctgcgtaccgccggtaaagtggcgatcaaactggttgacggcgatgagctgatcggcgttgacctgaccagcggcgaagacgaagtaatgctgttctccgctgaaggtaaagtggtgcgctttaaagagtcttctgtccgtgcgatgggctgcaacaccaccggtgttcgcggtattcgcttaggtgaaggcgataaagtcgtctctctgatcgtgcctcgtggcgatggcgcaatcctcaccgcaacgcaaaacggttacggtaaacgtaccgcagtggcggaatacccaaccaagtcgcgtgcgacgaaaggggttatctccatcaaggttaccgaacgtaacggtttagttgttggcgcggtacaggtagatgactgcgaccagatcatgatgatcaccgatgccggtacgctggtacgtactcgcgtttcggaaatcagcatcgtgggccgtaacacccagggcgtgatcctcatccgtactgcggaagatgaaaacgtagtgggtctgcaacgtgttgctgaaccggttgacgaggaagatctggataccatcgacggcagtgccgcggaaggggacgatgaaatcgctccggaagtggacgttgacgacgagccagaagaagaataa

SEQ ID NO: 5 - DNA, 2415 bp, synthetic construct
  source 1..2415: mol_type = other DNA
atgtcgaattcttatgactcctccagtatcaaagtcctgaaagggctggatgcggtgcgtaagcgcccgggtatgtatatcggcgacacggatgacggcaccggtctgcaccacatggtattcgatgtggtagataacgctatcgacgaagcgctcgccggtcactgtaaagaaattatcgtcaccattcacgccgataactctgtctctgtacaggatgacgggcgcggcattccgaccggtattcacccggaagagggcgtatcggcggcggaagtgatcatgaccgttctgcacgcaggcggtaaatttgacgataactcctataaagtgtccggcggtctgcacggcgttggtgtttcggtagtaaacgccctgtcgcaaaaactggagctggttatccagcgcgagggtaaaattcaccgtcagatctacgaacacggtgtaccgcaggccccgctggcggttaccggcgagactgaaaaaaccggcaccatggtgcgtttctggcccagcctcgaaaccttcaccaatgtgaccgagttcgaatatgaaattctggcgaaacgtctgcgtgagttgtcgttcctcaactccggcgtttccattcgtctgcgcgacaagcgcgacggcaaagaagaccacttccactatgaaggcggcatcaaggcgttcgttgaatatctgaacaagaacaaaacgccgatccacccgaatatcttctacttctccactgaaaaagacggtattggcgtcgaagtggcgttgcagtggaacgatggcttccaggaaaacatctactgctttaccaacaacattccgcagcgtgacggcggtactcacctggcaggcttccgtgcggcgatgacccgtaccctgaacgcctacatggacaaagaaggctacagcaaaaaagccaaagtcagcgccaccggtgacgatgcgcgtgaaggcctgattgcggtcgtttccgtgaaagtgccggacccgaaattctcctcccagaccaaagacaaactggtttcttctgaggtgaaatcggcggttgaacagcagatgaacgaactgctggcagaatacctgctggaaaacccaaccgacgcgaaaatcgtggttggcaaaattatcgatgctgcccgtgcccgtgaagcggcgcgtcgcgcgcgtgaaatgacccgccgtaaaggtgcgctcgacttagcgggcctgccgggcaaactggcagactgccaggaacgcgatccggcgctttccgaactgtacctggtggaaggggactccgcgggcggctctgcgaagcaggggcgtaaccgcaagaaccaggcgattctgccgctgaagggtaaaatcctcaacgtcgagaaagcgcgcttcgataagatgctctcttctcaggaagtggcgacgcttatcaccgcgcttggctgtggtatcggtcgtgacgagtacaacccggacaaactgcgttatcacagcatcatcatcatgaccgatgcggacgtcgacggctcgcacattcgtacgctgctgttgaccttcttctatcgtcagatgccggaaatcgttgaacgcggtcacgtctacatcgctcagccgccgctgtacaaagtgaagaaaggcaagcaggaacagtacattaaagacgacgaagcgatggatcagtaccagatctctatcgcgctggacggcgcaacgctgcacaccaacgccagtgcaccggcattggctggcgaagcgttagagaaactggtatctgagtacaacgcgacgcagaaaatgatcaatcgtatggagcgtcgttatccgaaagcaatgctgaaagagcttatctatcagccgacgttgacggaagctgacctttctgatgagcagaccgttacccgctgggtgaacgcgctggtcagcgaactgaacgacaaagaacagcacggcagccagtggaagtttgatgttcacaccaatgctgagcaaaacctgttcgagccgattgttcgcgtgcgtacccacggtgtggatactgactatccgctggatcacgagtttatcaccggtggcgaatatcgtcgtatctgcacgctgggtgagaaactgcgtggcttgctggaagaagatgcgtttatcgaacgtggcgagcgtcgtcagccggtagccagcttcgagcaggcgctggactggctggtgaaagagtcccgtcgcggcctctccatccagcgttataaaggtctgggcgagatgaacccggaacagctgtgggaaaccactatggacccggaaagtcgtcgtatgctgcgcgttaccgttaaagatgcgattgctgccgaccagttgttcaccacgctgatgggcgacgccgttgaaccgcgccgtgcgtttattgaagagaacgccctgaaagcggcgaatatcgatatttaa

SEQ ID NO: 6 - DNA, 2415 bp, synthetic construct
  source 1..2415: mol_type = other DNA
atgtcgaattcttatgactcctccagtatcaaagtcctgaaagggctggatgcggtgcgtaagcgcccgggtatgtatatcggcgacacggatgacggcaccggtctgcaccacatggtattcgaggtggtagataacgctatcgacgaagcgctcgcgggtcactgtaaagaaattatcgtcaccattcacgccgataactctgtctctgtacaggatgacgggcgcggcattccgaccggtattcacccggaagagggcgtatcggccgcggaagtgatcatgaccgttctgcacgcaggcggtaaatttgacgataactcctataaagtgtccggcggtctgcacggcgttggtgtttcggtagtaaacgccctgtcgcaaaaactggagctggttatccagtgcgagggtaaaattcaccgtcagatctacgaacacggtgtaccgcaggccccgctggcggttaccggcgagactgaaaaaaccggcaccatggtgcgtttctggcccagcctcgaaaccttcaccaatgtgaccgagttcgaatatgaaattctggcgaaacgtctgcgtgagttgtcgttcctcaactccggcgtttccattcgtctgcgcgacaagcgcgacggcaaagaagaccacttccactatgaaggcggcatcaaggcgttcgttgaatatctgaacaagaacaaaacgccgatccacccgaatatcttctacttctccactgaaaaagacggtattggcgtcgaagtggcgttgcagtggaacgatggcttccaggaaaacatctactgctttaccaacaacattccgcagcgtgacggcggtactcacctggcaggcttccgtgcggcgatgacccgtaccctgaacgcctacatggacaaagaaggctacagcaaaaaagccaaagtcagcgccaccggtgacgatgcgcgtgaaggcctgattgcggtcgtttccgtgaaagtgccggacccgaaattctcctcccagaccaaagacaaactggtttcttctgaggtgaaatcggcggttgaacagcagatgaacgaactgctggcagaatacctgctggaaaacccaaccgacgcgaaaatcgtggttggcaaaattatcgatgctgcccgtgcccgtgaagcggcgcgtcgcgcgcgtgaaatgacccgccgtaaaggtgcgctcgacttagcgggcctgccgggcaaactggcagactgccaggaacgcgatccggcgctttccgaactgtacctggtggaaggggactccgcgggcggctctgcgaagcaggggcgtaaccgcaagaaccaggcgattctgccgctgaagggtaaaatcctcaacgtcgagaaagcgcgcttcgataagatgctctcttctcaggaagtggcgacgcttatcaccgcgcttggctgtggtatcggtcgtgacgagtacaacccggacaaactgcgttatcacagcatcatcatcatgaccgatgcggacgtcgacggctcgcacattcgtacgctgctgttgaccttcttctatcgtcagatgccggaaatcgttgaacgcggtcacgtctacatcgctcagccgccgctgtacaaagtgaagaaaggcaagcaggaacagtacattaaagacgacgaagcgatggatcagtaccagatctctatcgcgctggacggcgcaacgctgcacaccaacgccagtgcaccggcattggctggcgaagcgttagagaaactggtatctgagtacaacgcgacgcagaaaatgatcaatcgtatggagcgtcgttatccgaaagcaatgctgaaagagcttatctatcagccgacgttgacggaagctgacctttctgatgagcagaccgttacccgctgggtgaacgcgctggtcagcgaactgaacgacaaagaacagcacggcagccagtggaagtttgatgttcacaccaatgctgagcaaaacctgttcgagccgattgttcgcgtgcgtacccacggtgtggatactgactatccgctggatcacgagtttatcaccggtggcgaatatcgtcgtatctgcacgctgggtgagaaactgcgtggcttgctggaagaagatgcgtttatcgaacgtggcgagcgtcgtcagccggtagccagcttcgagcaggcgctggactggctggtgaaagagtcccgtcgcggcctctccatccagcgttataaaggtctgggcgagatgaacccggaacagctgtgggaaaccactatggacccggaaagtcgtcgtatgctgcgcgttaccgttaaagatgcgattgctgccgaccagttgttcaccacgctgatgggcgacgccgttgaaccgcgccgtgcgtttattgaagagaacgccctgaaagcggcgaatatcgatatttaa

SEQ ID NO: 7 - DNA, 2415 bp, synthetic construct
  source 1..2415: mol_type = other DNA
atgtcgaattcttatgactcctccagtatcaaagtcctgaaagggctggatgcggtgcgtaagcgcccgggtatgtatatcggcgacacggatgacggcaccggtctgcaccacatggtattcgaggtggtagataacgctatcgacgaagcgctcgcgggtcactgtaaagaaattatcgtcaccattcacgccgataactctgtctctgtacaggatgacgggcgcggcattccgaccggtattcacccggaagagggcgtatcggcggcggaagtgatcatgaccgttctgcacgcaggcggtaaatttgacgataactcctataaagtgtccggcggtctgcacggcgttggtgtttcggtagtaaacgccctgtcgcaaaaactggagctggttatccagcgcgagggtaaaattcaccgtcagatctacgaacacggtgtaccgcaggccccgctggcggttaccggcgagactgaaaaaaccggcaccatggtgcgtttctggcccagcctcgaaaccttcaccaatgtgaccgagttcgaatatgaaattctggcgaaacgtctgcgtgagttgtcgttcctcaactccggcgtttccattcgtctgcgcgacaagcgcgacggcaaagaagaccacttccactatgaaggcggcatcaaggcgttcgttgaatatctgaacaagaacaaaacgccgatccacccgaatatcttctacttctccactgaaaaagacggtattggcgtcgaagtggcgttgcagtggaacgatggcttccaggaaaacatctactgctttaccaacaacattccgcagcgtgacggcggtactcacctggcaggcttccgtgcggcgatgacccgtaccctgaacgcctacatggacaaagaaggctacagcaaaaaagccaaagtcagcgccaccggtgacgatgcgcgtgaaggcctgattgcggtcgtttccgtgaaagtgccggacccgaaattctcctcccagaccaaagacaaactggtttcttctgaggtgaaatcggcggttgaacagcagatgaacgaactgctggcagaatacctgctggaaaacccaaccgacgcgaaaatcgtggttggcaaaattatcgatgctgcccgtgcccgtgaagcggcgcgtcgcgcgcgtgaaatgacccgccgtaaaggtgcgctcgacttagcgggcctgccgggcaaactggcagactgccaggaacgcgatccggcgctttccgaactgtacctggtggaaggggactccgcgggcggctctgcgaagcaggggcgtaaccgcaagaaccaggcgattctgccgctgaagggtaaaatcctcaacgtcgagaaagcgcgcttcgataagatgctctcttctcaagaagtggcgacgcttatcaccgcgcttggctgtggtatcggtcgtgacgagtacaacccggacaaactgcgttatcacagcatcatcatcatgaccgccgcggacgtcgacggctcgcacattcgtacgctgctgttgaccttcttctatcgtcagatgccggaaatcgttgaacgcggtcacgtctacatcgctcagccgccgctgtacaaagtgaagaaaggcaagcaggaacagtacattaaagacgacgaagcgatggatcagtaccagatctctatcgcgctggacggcgcaacgctgcacaccaacgccagtgcaccggcattggctggcgaagcgttagagaaactggtatctgagtacaacgcgacgcagaaaatgatcaatcgtatggagcgtcgttatccgaaagcaatgctgaaagagcttatctatcagccgacgttgacggaagctgacctttctgatgagcagaccgttacccgctgggtgaacgcgctggtcagcgaactgaacgacaaagaacagcacggcagccagtggaagtttgatgttcacaccaatgctgagcaaaacctgttcgagccgattgttcgcgtgcgtacccacggtgtggatactgactatccgctggatcacgagtttatcaccggtggcgaatatcgtcgtatctgcacgctgggtgagaaactgcgtggcttgctggaagaagatgcgtttatcgaacgtggcgagcgtcgtcagccggtagccagcttcgagcaggcgctggactggctggtgaaagagtcccgtcgcggcctctccatccagcgttataaaggtctgggcgagatgaacccggaacagctgtgggaaaccactatggacccggaaagtcgtcgtatgctgcgcgttaccgttaaagatgcgattgctgccgaccagttgttcaccacgctgatgggcgacgccgttgaaccgcgccgtgcgtttattgaagagaacgccctgaaagcggcgaatatcgatatttaa

SEQ ID NO: 8 - DNA, 20 bp, synthetic construct
  source 1..20: mol_type = other DNA
ctatctggattatgcgatgt

SEQ ID NO: 9 - DNA, 20 bp, synthetic construct
  source 1..20: mol_type = other DNA
caacagcgcagacatcaacc

SEQ ID NO: 10 - DNA, 20 bp, synthetic construct
  source 1..20: mol_type = other DNA
cgctatcgacgaagcgctcg

SEQ ID NO: 11 - DNA, 20 bp, synthetic construct
  source 1..20: mol_type = other DNA
cccggaagagggcgtatcgg

SEQ ID NO: 12 - DNA, 20 bp, synthetic construct
  source 1..20: mol_type = other DNA
cgataagatgctctcttctc

SEQ ID NO: 13 - DNA, 1000 bp, synthetic construct
  source 1..1000: mol_type = other DNA
gcggtttgaactcaccttccagatcccaccagcgggaggcgacggcttcaaatttagcgatctcttcgtggtctacgttatggtttaccggcgatttttcggcattcattggcacttctactccgtaattggcaagacaaacgagtatatcaggcattggatgtgaataaagcgtataggtttacctcaaactgcgcggctgtgttataatttgcgacctttgaatccgggatacagtagagggatagcggttagatgagcgaccttgcgagagaaattacaccggtcaacattgaggaagagctgaagagctcctatctggattatgcgatgtctgtcattgttggccgtgcgctgccagatgtccgagatggcctgaagccggtacaccgtcgcgtactttacgccatgaacgtactaggcaatgactggaacaaagcctataaaaaatctgcccgtgtcgttggtgacgtaatcggtaaataccatcccgcaggtgactcggcggtctatgacacgatcgtccgcatggcgcagccattctcgctgcgttatatgctggtagacggtcagggtaacttcggttctatcgacggcgactctgcggcggcaatgcgttatacggaaatccgtctggcgaaaattgcccatgaactgatggccgatctcgaaaaagagacggtcgatttcgttgataactatgacggcacggaaaaaattccggacgtcatgccaaccaaaattcctaacctgctggtgaacggttcttccggtatcgccgtaggtatggcaaccaacatcccgccgcacaacctgacggaagtcatcaacggttgtctggcgtatattgatgatgaagacatcagcattgaagggctgatggaacacatcccggggccggacttcccgacggcggcaatcattaacggtcgtcgcggtattgaagaagcttaccgtaccggtcgcggcaaggtgtatatccgcgctcgcgcagaagtgg

SEQ ID NO: 14 - DNA, 1000 bp, synthetic construct
  source 1..1000: mol_type = other DNA
gttcggcgtgcgtgatggtctgtactacctgaccgaacagcaagctcaggcgattctggatctgcgtttgcagaaactgaccggtcttgagcacgaaaaactgctcgacgaatacaaagagctgctggatcagatcgcggaactgttgcgtattcttggtagcgccgatcgtctgatggaagtgatccgtgaagagctggagctggttcgtgaacagttcggtgacaaacgtcgtactgaaatcaccgccaacagcgcagacatcaacctcgaagatctgatcacccaggaagatgtggtcgtgacgctctctcaccagggctacgttaagtatcagccgctttctgaatacgaagcgcagcgtcgtggcgggaaaggtaaatctactgcacgtattaaagaagaagactttatcgaccgactgctggtggcgaacgcccacgaccatattctgtgcttctccagccgtggtcgcgtctattcgatgaaagtttatcagttgccggaagccactcgtggcgcgcgcggtcgtccgatcgtcaacctgctgccgctggagcaggacgaacgtatcactgcgatcctgccagtgaccgagtttgaagaaggcgtgaaagtcttcatggcgaccgctaacggtaccgtgaagaaaactgtcctcaccgagttcaaccgtctgcgtaccgccggtaaagtggcgatcaaactggttgacggcgatgagctgatcggcgttgacctgaccagcggcgaagacgaagtaatgctgttctccgctgaaggtaaagtggtgcgctttaaagagtcttctgtccgtgcgatgggctgcaacaccaccggtgttcgcggtattcgcttaggtgaaggcgataaagtcgtctctctgatcgtgcctcgtggcgatggcgcaatcctcaccgcaacgcaaaacggttacggtaaacgtaccgcagtggcggaatacccaaccaagtcgcgtgcgacgaaaggggttatctcc

SEQ ID NO: 15 - DNA, 1000 bp, synthetic construct
  source 1..1000: mol_type = other DNA
cgacggtgcgccggtggaagataccttatcgcgtgggcagcttaagctgttgatgtgcgccttacgtctggcgcaaggagagttcctcacccgtgaaagcgggcggcggtgtctctacctgatagatgattttgcctctgagcttgatgatgagcgtcgcgggctgcttgccagccgcttaaaagcgacgcaatcacaggtctttgtcagcgcgatcagtgctgaacacgttatagacatgtcggacgaaaattcgaagatgtttaccgtggaaaagggtaaaataacggattaacccaagtataaatgagcgagaaacgttgatgtcgaattcttatgactcctccagtatcaaagtcctgaaagggctggatgcggtgcgtaagcgcccgggtatgtatatcggcgacacggatgacggcaccggtctgcaccacatggtattcgatgtggtagataacgctatcgacgaagcgctcgccggtcactgtaaagaaattatcgtcaccattcacgccgataactctgtctctgtacaggatgacgggcgcggcattccgaccggtattcacccggaagagggcgtatcggcggcggaagtgatcatgaccgttctgcacgcaggcggtaaatttgacgataactcctataaagtgtccggcggtctgcacggcgttggtgtttcggtagtaaacgccctgtcgcaaaaactggagctggttatccagcgcgagggtaaaattcaccgtcagatctacgaacacggtgtaccgcaggccccgctggcggttaccggcgagactgaaaaaaccggcaccatggtgcgtttctggcccagcctcgaaaccttcaccaatgtgaccgagttcgaatatgaaattctggcgaaacgtctgcgtgagttgtcgttcctcaactccggcgtttccattcgtctgcgcgacaagcgcgacggcaaagaagaccacttccactatgaaggcggcatcaaggcgttcgt

SEQ ID NO: 16 - DNA, 1000 bp, synthetic construct
  source 1..1000: mol_type = other DNA
cgttgatgtcgaattcttatgactcctccagtatcaaagtcctgaaagggctggatgcggtgcgtaagcgcccgggtatgtatatcggcgacacggatgacggcaccggtctgcaccacatggtattcgaggtggtagataacgctatcgacgaagcgctcgcgggtcactgtaaagaaattatcgtcaccattcacgccgataactctgtctctgtacaggatgacgggcgcggcattccgaccggtattcacccggaagagggcgtatcggccgcggaagtgatcatgaccgttctgcacgcaggcggtaaatttgacgataactcctataaagtgtccggcggtctgcacggcgttggtgtttcggtagtaaacgccctgtcgcaaaaactggagctggttatccagtgcgagggtaaaattcaccgtcagatctacgaacacggtgtaccgcaggccccgctggcggttaccggcgagactgaaaaaaccggcaccatggtgcgtttctggcccagcctcgaaaccttcaccaatgtgaccgagttcgaatatgaaattctggcgaaacgtctgcgtgagttgtcgttcctcaactccggcgtttccattcgtctgcgcgacaagcgcgacggcaaagaagaccacttccactatgaaggcggcatcaaggcgttcgttgaatatctgaacaagaacaaaacgccgatccacccgaatatcttctacttctccactgaaaaagacggtattggcgtcgaagtggcgttgcagtggaacgatggcttccaggaaaacatctactgctttaccaacaacattccgcagcgtgacggcggtactcacctggcaggcttccgtgcggcgatgacccgtaccctgaacgcctacatggacaaagaaggctacagcaaaaaagccaaagtcagcgccaccggtgacgatgcgcgtgaaggcctgattgcggtcgtttccgtgaaagtgccggacccgaaatt

SEQ ID NO: 17 - DNA, 1000 bp, synthetic construct
  source 1..1000: mol_type = other DNA
tgaacgaactgctggcagaatacctgctggaaaacccaaccgacgcgaaaatcgtggttggcaaaattatcgatgctgcccgtgcccgtgaagcggcgcgtcgcgcgcgtgaaatgacccgccgtaaaggtgcgctcgacttagcgggcctgccgggcaaactggcagactgccaggaacgcgatccggcgctttccgaactgtacctggtggaaggggactccgcgggcggctctgcgaagcaggggcgtaaccgcaagaaccaggcgattctgccgctgaagggtaaaatcctcaacgtcgagaaagcgcgcttcgataagatgctctcttctcaagaagtggcgacgcttatcaccgcgcttggctgtggtatcggtcgtgacgagtacaacccggacaaactgcgttatcacagcatcatcatcatgaccgccgcggacgtcgacggctcgcacattcgtacgctgctgttgaccttcttctatcgtcagatgccggaaatcgttgaacgcggtcacgtctacatcgctcagccgccgctgtacaaagtgaagaaaggcaagcaggaacagtacattaaagacgacgaagcgatggatcagtaccagatctctatcgcgctggacggcgcaacgctgcacaccaacgccagtgcaccggcattggctggcgaagcgttagagaaactggtatctgagtacaacgcgacgcagaaaatgatcaatcgtatggagcgtcgttatccgaaagcaatgctgaaagagcttatctatcagccgacgttgacggaagctgacctttctgatgagcagaccgttacccgctgggtgaacgcgctggtcagcgaactgaacgacaaagaacagcacggcagccagtggaagtttgatgttcacaccaatgctgagcaaaacctgttcgagccgattgttcgcgtgcgtacccacggtgtggatactgactatccgctggatcacgagtttatcaccggtggcga

SEQ ID NO: 18 - DNA, 27 bp, synthetic construct
  source 1..27: mol_type = other DNA
gcatgacaccggacattatcctgcagc

SEQ ID NO: 19 - DNA, 27 bp, synthetic construct
  source 1..27: mol_type = other DNA
tccccaaatacaaaaccaatttcagcc

SEQ ID NO: 20 - DNA, 25 bp, synthetic construct
  source 1..25: mol_type = other DNA
catcatactgcccggcatgttttgc

SEQ ID NO: 21 - DNA, 26 bp, synthetic construct
  source 1..26: mol_type = other DNA
cggcatcggtgatcatcatgatctgg

SEQ ID NO: 22 - DNA, 27 bp, synthetic construct
  source 1..27: mol_type = other DNA
ctcgcgatcgtgctcatatccttgaag

SEQ ID NO: 23 - DNA, 27 bp, synthetic construct
  source 1..27: mol_type = other DNA
acacgttgcagacccactacgttttca

SEQ ID NO: 24 - DNA, 29 bp, synthetic construct
  source 1..29: mol_type = other DNA
gatttttcaccgcctggagcaatctcaag

SEQ ID NO: 25 - DNA, 32 bp, synthetic construct
  source 1..32: mol_type = other DNA
aagcgttacgtgttgacccaaaaagtatagat

SEQ ID NO: 26 - DNA, 32 bp, synthetic construct
  source 1..32: mol_type = other DNA
tagatgattttgcctctgagcttgatgatgag

SEQ ID NO: 27 - DNA, 32 bp, synthetic construct; identical to SEQ ID NO: 25
  source 1..32: mol_type = other DNA

SEQ ID NO: 28 - DNA, 32 bp, synthetic construct; identical to SEQ ID NO: 26
  source 1..32: mol_type = other DNA

SEQ ID NO: 29 - DNA, 32 bp, synthetic construct; identical to SEQ ID NO: 25
  source 1..32: mol_type = other DNA

SEQ ID NO: 30 - DNA, 80 bp, synthetic construct
  source 1..80: mol_type = other DNA
aaaaaaaaaaaaaaaaaaaaaaaaaaaaaaaaaaaaaaaaaaaaaaaaaaaaaaaaaaaaaaaaaaaaaaaaaaaaaaaa

SEQ ID NO: 31 - DNA, 100 bp, synthetic construct
  source 1..100: mol_type = other DNA
aaaaaaaaaaaaaaaaaaaaaaaaaaaaaaaaaaaaaaaaaaaaaaaaaaaaaaaaaaaaaaaaaaaaaaaaaaaaaaaaaaaaaaaaaaaaaaaaaaaa

SEQ ID NO: 32 - DNA, 120 bp, synthetic construct
  source 1..120: mol_type = other DNA
aaaaaaaaaaaaaaaaaaaaaaaaaaaaaaaaaaaaaaaaaaaaaaaaaaaaaaaaaaaaaaaaaaaaaaaaaaaaaaaaaaaaaaaaaaaaaaaaaaaaaaaaaaaaaaaaaaaaaaaa

SEQ ID NO: 33 - DNA, 110 bp, synthetic construct
  source 1..110: mol_type = other DNA
aaaaaaaaaaaaaaaaaaaaaaaaaaaaaagcatatgactaaaaaaaaaaaaaaaaaaaaaaaaaaaaaaaaaaaaaaaaaaaaaaaaaaaaaaaaaaaaaaaaaaaaaa

SEQ ID NO: 34 - DNA, 123 bp, synthetic construct
  source 1..123: mol_type = other DNA
aaaaaaaaaaaaaaaaaaaaaaaaaaaaaagcatatgactaaaaaaaaaaaaaaaaaaaaaaaaaaaaaagcatatgactaaaaaaaaaaaaaaaaaaaaaaaaaaaaaaaaaaaaaaaaaaa

SEQ ID NO: 35 - DNA, 991 bp, synthetic construct
  source 1..991: mol_type = other DNA
taatacgactcactataaggggtcttctggtccccacagactcagagagaacccgccaccatggtgagcaagggcgaggagctgttcaccggggtggtgcccatcctggtcgagctggacggcgacgtaaacggccacaagttcagcgtgtccggcgagggcgagggcgatgccacctacggcaagctgaccctgaagttcatctgcaccaccggcaagctgcccgtgccctggcccaccctcgtgaccaccctgacctacggcgtgcagtgcttcagccgctaccccgaccacatgaagcagcacgacttcttcaagtccgccatgcccgaaggctacgtccaggagcgcaccatcttcttcaaggacgacggcaactacaagacccgcgccgaggtgaagttcgagggcgacaccctggtgaaccgcatcgagctgaagggcatcgacttcaaggaggacggcaacatcctggggcacaagctggagtacaactacaacagccacaacgtctatatcatggccgacaagcagaagaacggcatcaaggtgaacttcaagatccgccacaacatcgaggacggcagcgtgcagctcgccgaccactaccagcagaacacccccatcggcgacggccccgtgctgctgcccgacaaccactacctgagcacccagtccgccctgagcaaagaccccaacgagaagcgcgatcacatggtcctgctggagttcgtgaccgccgccgggatcactctcggcatggacgagctgtacaagtaatagtaagctggagcctcggtggccatgcttcttgccccttgggcctccccccagcccctcctccccttcctgcacccgtacccccgtggtctttgaataaagtctgagtgggcggcaactagtaaaaaaaaaaaaaaaaaaaaaaaaaaaaaaaaaaaaaaaaaaaaaaaaaaaaaaaaaaaaaaaaaaaaaaaaaaaaaaaaggaagagc

SEQ ID NO: 36 - DNA, 2999 bp, synthetic construct
  source 1..2999: mol_type = other DNA
gactcttcgcgatgtacgggccagatatacgcgttgacattgattattgactagttattaatagtaatcaattacggggtcattagttcatagcccatatatggagttccgcgttacataacttacggtaaatggcccgcctggctgaccgcccaacgacccccgcccattgacgtcaataatgacgtatgttcccatagtaacgccaatagggactttccattgacgtcaatgggtggactatttacggtaaactgcccacttggcagtacatcaagtgtatcatatgccaagtacgccccctattgacgtcaatgacggtaaatggcccgcctggcattatgcccagtacatgaccttatgggactttcctacttggcagtacatctacgtattagtcatcgctattaccatggtgatgcggttttggcagtacatcaatgggcgtggatagcggtttgactcacggggatttccaagtctccaccccattgacgtcaatgggagtttgttttggcaccaaaatcaacgggactttccaaaatgtcgtaacaactccgccccattgacgcaaatgggcggtaggcgtgtacggtgggaggtctatataagcagagctctctggctaactagagaacccactgcttactggcttatcgaaattaatacgactcactatagggagacccaagctggctagcgtttaaacttaagcttggtaccgagctcggatccactagtccagtgtggtggaattctgcagatatccagcacagtggcggccgctcgagtctagagggcccgtttaaacccgctgatcagcctcgactgtgccttctagttgccagccatctgttgtttgcccctcccccgtgccttccttgaccctggaaggtgccactcccactgtcctttcctaataaaatgaggaaattgcatcgcattgtctgagtaggtgtcattctattctggggggtggggtggggcaggacagcaagggggaggattgggaagacaatagcaggcatgctggggatgcggtgggctctatggcttctactgggcggttttatggacagcaagcgaaccggaattgccagctggggcgccctctggtaaggttgggaagccctgcaaagtaaactggatggctttctcgccgccaaggatctgatggcgcaggggatcaagctctgatcaagagacaggatgaggatcgtttcgcatgattgaacaagatggattgcacgcaggttctccggccgcttgggtggagaggctattcggctatgactgggcacaacagacaatcggctgctctgatgccgccgtgttccggctgtcagcgcaggggcgcccggttctttttgtcaagaccgacctgtccggtgccctgaatgaactgcaagacgaggcagcgcggctatcgtggctggccacgacgggcgttccttgcgcagctgtgctcgacgttgtcactgaagcgggaagggactggctgctattgggcgaagtgccggggcaggatctcctgtcatctcaccttgctcctgccgagaaagtatccatcatggctgatgcaatgcggcggctgcatacgcttgatccggctacctgcccattcgaccaccaagcgaaacatcgcatcgagcgagcacgtactcggatggaagccggtcttgtcgatcaggatgatctggacgaagagcatcaggggctcgcgccagccgaactgttcgccaggctcaaggcgagcatgcccgacggcgaggatctcgtcgtgacccatggcgatgcctgcttgccgaatatcatggtggaaaatggccgcttttctggattcatcgactgtggccggctgggtgtggcggaccgctatcaggacatagcgttggctacccgtgatattgctgaagagcttggcggcgaatgggctgaccgcttcctcgtgctttacggtatcgccgctcccgattcgcagcgcatcgccttctatcgccttcttgacgagttcttctgaattattaacgcttacaatttcctgatgcggtattttctccttacgcatctgtgcggtatttcacaccgcatacaggtggcacttttcggggaaatgtgcgcggaacccctatttgtttatttttctaaatacattcaaatatgtatccgctcatgagacaataaccctgataaatgcttcaataatagcacgtgctaaaacttcatttttaatttaaaaggatctaggtgaagatcctttttgataatctcatgaccaaaatcccttaacgtgagttttcgttccactgagcgtcagaccccgtagaaaagatcaaaggatcttcttgagatcctttttttctgcgcgtaatctgctgcttgcaaacaaaaaaaccaccgctaccagcggtggtttgtttgccggatcaagagctaccaactctttttccgaaggtaactggcttcagcagagcgcagataccaaatactgtccttctagtgtagccgtagttaggccaccacttcaagaactctgtagcaccgcctacatacctcgctctgctaatcctgttaccagtggctgctgccagtggcgataagtcgtgtcttaccgggttggactcaagacgatagttaccggataaggcgcagcggtcgggctgaacggggggttcgtgcacacagcccagcttggagcgaacgacctacaccgaactgagatacctacagcgtgagctatgagaaagcgccacgcttcccgaagggagaaaggcggacaggtatccggtaagcggcagggtcggaacaggagagcgcacgagggagcttccagggggaaacgcctggtatctttatagtcctgtcgggtttcgccacctctgacttgagcgtcgatttttgtgatgctcgtcaggggggcggagcctatggaaaaacgccagcaacgcggcctttttacggttcctgggcttttgctggccttttgctcacatgttctt

SEQ ID NO: 37 - protein, 875 aa, Escherichia coli
MSDLAREITPVNIEEELKSSYLDYAMSVIVGRALPDVRDGLKPVHRRVLYAMNVLGNDWNKAYKKSARVVGDVIGKYHPHGDSAVYDTIVRMAQPFSLRYMLVDGQGNFGSIDGDSAAAMRYTEIRLAKIAHELMADLEKETVDFVDNYDGTEKIPDVMPTKIPNLLVNGSSGIAVGMATNIPPHNLTEVINGCLAYIDDEDISIEGLMEHIPGPDFPTAAIINGRRGIEEAYRTGRGKVYIRARAEVEVDAKTGRETIIVHEIPYQVNKARLIEKIAELVKEKRVEGISALRDESDKDGMRIVIEVKRDAVGEVVLNNLYSQTQLQVSFGINMVALHHGQPKIMNLKDIIAAFVRHRREVVTRRTIFELRKARDRAHILEALAVALANIDPIIELIRHAPTPAEAKTALVANPWQLGNVAAMLERAGDDAARPEWLEPEFGVRDGLYYLTEQQAQAILDLRLQKLTGLEHEKLLDEYKELLDQIAELLRILGSADRLMEVIREELELVREQFGDKRRTEITANSADINLEDLITQEDVVVTLSHQGYVKYQPLSEYEAQRRGGKGKSAARIKEEDFIDRLLVANTHDHILCFSSRGRVYSMKVYQLPEATRGARGRPIVNLLPLEQDERITAILPVTEFEEGVKVFMATANGTVKKTVLTEFNRLRTAGKVAIKLVDGDELIGVDLTSGEDEVMLFSAEGKVVRFKESSVRAMGCNTTGVRGIRLGEGDKVVSLIVPRGDGAILTATQNGYGKRTAVAEYPTKSRATKGVISIKVTERNGLVVGAVQVDDCDQIMMITDAGTLVRTRVSEISIVGRNTQGVILIRTAEDENVVGLQRVAEPVDEEDLDTIDGSAAEGDDEIAPEVDVDDEPEEE

SEQ ID NO: 38 - protein, 875 aa, synthetic construct
  VARIANT 80: note = H or A
  VARIANT 569: note = A or T
  VARIANT 586: note = T or A
MSDLAREITPVNIEEELKSSYLDYAMSVIVGRALPDVRDGLKPVHRRVLYAMNVLGNDWNKAYKKSARVVGDVIGKYHPXGDSAVYDTIVRMAQPFSLRYMLVDGQGNFGSIDGDSAAAMRYTEIRLAKIAHELMADLEKETVDFVDNYDGTEKIPDVMPTKIPNLLVNGSSGIAVGMATNIPPHNLTEVINGCLAYIDDEDISIEGLMEHIPGPDFPTAAIINGRRGIEEAYRTGRGKVYIRARAEVEVDAKTGRETIIVHEIPYQVNKARLIEKIAELVKEKRVEGISALRDESDKDGMRIVIEVKRDAVGEVVLNNLYSQTQLQVSFGINMVALHHGQPKIMNLKDIIAAFVRHRREVVTRRTIFELRKARDRAHILEALAVALANIDPIIELIRHAPTPAEAKTALVANPWQLGNVAAMLERAGDDAARPEWLEPEFGVRDGLYYLTEQQAQAILDLRLQKLTGLEHEKLLDEYKELLDQIAELLRILGSADRLMEVIREELELVREQFGDKRRTEITANSADINLEDLITQEDVVVTLSHQGYVKYQPLSEYEAQRRGGKGKSXARIKEEDFIDRLLVANXHDHILCFSSRGRVYSMKVYQLPEATRGARGRPIVNLLPLEQDERITAILPVTEFEEGVKVFMATANGTVKKTVLTEFNRLRTAGKVAIKLVDGDELIGVDLTSGEDEVMLFSAEGKVVRFKESSVRAMGCNTTGVRGIRLGEGDKVVSLIVPRGDGAILTATQNGYGKRTAVAEYPTKSRATKGVISIKVTERNGLVVGAVQVDDCDQIMMITDAGTLVRTRVSEISIVGRNTQGVILIRTAEDENVVGLQRVAEPVDEEDLDTIDGSAAEGDDEIAPEVDVDDEPEEE

SEQ ID NO: 39 - protein, 804 aa, Escherichia coli
MSNSYDSSSIKVLKGLDAVRKRPGMYIGDTDDGTGLHHMVFEVVDNAIDEALAGHCKEIIVTIHADNSVSVQDDGRGIPTGIHPEEGVSAAEVIMTVLHAGGKFDDNSYKVSGGLHGVGVSVVNALSQKLELVIQREGKIHRQIYEHGVPQAPLAVTGETEKTGTMVRFWPSLETFTNVTEFEYEILAKRLRELSFLNSGVSIRLRDKRDGKEDHFHYEGGIKAFVEYLNKNKTPIHPNIFYFSTEKDGIGVEVALQWNDGFQENIYCFTNNIPQRDGGTHLAGFRAAMTRTLNAYMDKEGYSKKAKVSATGDDAREGLIAVVSVKVPDPKFSSQTKDKLVSSEVKSAVEQQMNELLAEYLLENPTDAKIVVGKIIDAARAREAARRAREMTRRKGALDLAGLPGKLADCQERDPALSELYLVEGDSAGGSAKQGRNRKNQAILPLKGKILNVEKARFDKMLSSQEVATLITALGCGIGRDEYNPDKLRYHSIIIMTDADVDGSHIRTLLLTFFYRQMPEIVERGHVYIAQPPLYKVKKGKQEQYIKDDEAMDQYQISIALDGATLHTNASAPALAGEALEKLVSEYNATQKMINRMERRYPKAMLKELIYQPTLTEADLSDEQTVTRWVNALVSELNDKEQHGSQWKFDVHTNAEQNLFEPIVRVRTHGVDTDYPLDHEFITGGEYRRICTLGEKLRGLLEEDAFIERGERRQPVASFEQALDWLVKESRRGLSIQRYKGLGEMNPEQLWETTMDPESRRMLRVTVKDAIAADQLFTTLMGDAVEPRRAFIEENALKAANIDI

SEQ ID NO: 40 - protein, 804 aa, synthetic construct
  VARIANT 42: note = E or D
  VARIANT 136: note = R or C
  VARIANT 498: note = D or A
MSNSYDSSSIKVLKGLDAVRKRPGMYIGDTDDGTGLHHMVFXVVDNAIDEALAGHCKEIIVTIHADNSVSVQDDGRGIPTGIHPEEGVSAAEVIMTVLHAGGKFDDNSYKVSGGLHGVGVSVVNALSQKLELVIQXEGKIHRQIYEHGVPQAPLAVTGETEKTGTMVRFWPSLETFTNVTEFEYEILAKRLRELSFLNSGVSIRLRDKRDGKEDHFHYEGGIKAFVEYLNKNKTPIHPNIFYFSTEKDGIGVEVALQWNDGFQENIYCFTNNIPQRDGGTHLAGFRAAMTRTLNAYMDKEGYSKKAKVSATGDDAREGLIAVVSVKVPDPKFSSQTKDKLVSSEVKSAVEQQMNELLAEYLLENPTDAKIVVGKIIDAARAREAARRAREMTRRKGALDLAGLPGKLADCQERDPALSELYLVEGDSAGGSAKQGRNRKNQAILPLKGKILNVEKARFDKMLSSQEVATLITALGCGIGRDEYNPDKLRYHSIIIMTXADVDGSHIRTLLLTFFYRQMPEIVERGHVYIAQPPLYKVKKGKQEQYIKDDEAMDQYQISIALDGATLHTNASAPALAGEALEKLVSEYNATQKMINRMERRYPKAMLKELIYQPTLTEADLSDEQTVTRWVNALVSELNDKEQHGSQWKFDVHTNAEQNLFEPIVRVRTHGVDTDYPLDHEFITGGEYRRICTLGEKLRGLLEEDAFIERGERRQPVASFEQALDWLVKESRRGLSIQRYKGLGEMNPEQLWETTMDPESRRMLRVTVKDAIAADQLFTTLMGDAVEPRRAFIEENALKAANIDI

SEQ ID NO: 41 - DNA, 1830 bp, Escherichia coli
  source 1..1830: mol_type = genomic DNA
gtggcgcaggcggaagtgttgaatctggagtccggagctaaacaggttttacaagaaacctttggctaccaacagtttcgccccggccaggaagaaattatcgacactgtgctttccggccgcgattgcctcgtcgtcatgcccactggtggcggaaaatccctttgctatcaaatccctgccttattgctaaacggccttaccgtggttgtttcaccgctgatttcgttgatgaaagatcaggtggatcaactgcaagccaacggcgtggcggcggcgtgccttaactcgacgcaaacccgcgaacagcaacttgaagtgatgacaggctgccgcaccgggcaaattcgtctgctttatatcgccccggaacgcctgatgctggataactttcttgagcatctggcgcactggaatccggtgttattagccgttgatgaagcgcactgtatctcccaatggggccacgatttccgcccggaatatgccgcgctcggtcagttgcgccagcggttcccgacgctgccgtttatggcgctgaccgccacagccgacgacaccacgcgccaggatatcgtgcgcctgctggggctgaacgatccgctgattcaaatcagcagttttgaccgtccgaatattcgctacatgctgatggagaagttcaaaccgctcgatcagttgatgcgctacgtgcaggaacagcgcggtaagtcaggcattatctactgcaacagccgcgcgaaagtagaagacaccgctgcgcgcctgcaaagcaagggaattagcgcggcggcctatcatgccgggctggaaaataatgttcgcgccgatgtgcaggaaaaattccagcgcgatgacctgcaaattgtggtggcgacggtggcgttcggcatgggcatcaataaaccaaacgttcgcttcgtggtccactttgatattccgcgcaatatcgaatcctattatcaggaaaccggacgcgccgggcgtgatggcctgcccgcggaagcgatgctgttttacgatccggctgatatggcgtggctgcgccgttgtctggaagagaagccgcaggggcagttgcaggatatcgagcgccacaaactcaatgcgatgggcgcgtttgccgaagcgcaaacttgccgtcgtctggtattgctgaactattttggcgaagggcgtcaggagccgtgcgggaactgcgatatctgcctcgatccgccgaaacagtacgacggttcaaccgatgctcagattgccctttccaccattggtcgtgtgaatcagcggtttgggatgggttatgtggtggaagtgattcgtggtgctaataaccagcgtatccgcgactatggtcatgacaaactgaaagtctatggcatgggccgtgataaaagccatgaacattgggtgagcgtgatccgccagctgattcacctcggcctggtgacgcaaaatattgcccagcattctgccctacaactgacagaggccgcgcgcccggtgctgcgcggcgaatcctctttgcaacttgccgtgccgcgtatcgtggcgctcaaaccgaaagcgatgcagaaatcgttcggcggcaactatgatcgcaaactgttcgccaaattacgcaaactgcgtaaatcgatagccgatgaaagtaatgtcccgccgtacgtggtgtttaacgacgcaaccttgattgagatggctgaacagatgccgatcaccgccagcgaaatgctcagcgttaacggcgttgggatgcgcaagctggaacgctttggcaaaccgtttatggcgctgattcgtgcgcatgttgatggcgatgacgaagagtag

SEQ ID NO: 42 - DNA, 1413 bp, synthetic construct
  source 1..1413: mol_type = other DNA
gacaccatcgaatggtgcaaaacctttcgcggtatggcatgatagcgcccggaagagagtcaattcagggtggtgaatgtgaaaccagtaacgttatacgatgtcgcagagtatgccggtgtctcttatcagaccgtttcccgcgtggtgaaccaggccagccacgtttctgcgaaaacgcgggaaaaagtggaagcggcgatggcggagctgaattacattcccaaccgcgtggcacaacaactggcgggcaaacagtcgttgctgattggcgttgccacctccagtctggccctgcacgcgccgtcgcaaattgtcgcggcgattaaatctcgcgccgatcaactgggtgccagcgtggtggtgtcgatggtagaacgaagcggcgtcgaagcctgtaaagcggcggtgcacaatcttctcgcgcaacgcgtcagtgggctgatcattaactatccgctggatgaccaggatgccattgctgtggaagctgcctgcactaatgttccggcgttatttcttgatgtctctgaccagacacccatcaacagtattattttctcccatgaagacggtacgcgactgggcgtggagcatctggtcgcattgggtcaccagcaaatcgcgctgttagcgggcccattaagttctgtctcggcgcgtctgcgtctggctggctggcataaatatctcactcgcaatcaaattcagccgatagcggaacgggaaggcgactggagtgccatgtccggttttcaacaaaccatgcaaatgctgaatgagggcatcgttcccactgcgatgctggttgccaacgatcagatggcgctgggcgcaatgcgcgccattaccgagtccgggctgcgcgttggtgcggatatctcggtagtgggatacgacgataccgaagacagctcatgttatatcccgccgttaaccaccatcaaacaggattttcgcctgctggggcaaaccagcgtggaccgcttgctgcaactctctcagggccaggcggtgaagggcaatcagctgttgcccgtctcactggtgaaaagaaaaaccaccctggcgcccaatacgcaaaccgcctctccccgcgcgttggccgattcattaatgcagctggcacgacaggtttcccgactggaaagcgggcagtgaaattcgcgcaacgcaattaatgtaagttagctcactcattaggcaccaaataaaacgaaaggctcagtcgaaagactgggcctttcgttttatctgttgtttgtcggtgaacgctctcctgagtaggacaaatccgccgggagcggatttgaacgttgcgaagcaacggcccggagggtggcgggcaggacgcccgccataaactgccaggcatcaaattaagcagaaggccatcctgacggatggcctttt

SEQ ID NO: 43 - DNA, 1062 bp, Escherichia coli
  source 1..1062: mol_type = genomic DNA
atggctatcgacgaaaacaaacagaaagcgttggcggcagcactgggccagattgagaaacaatttggtaaaggctccatcatgcgcctgggtgaagaccgttccatggatgtggaaaccatctctaccggttcgctttcactggatatcgcgcttggggcaggtggtctgccgatgggccgtatcgtcgaaatctacggaccggaatcttccggtaaaaccacgctgacgctgcaggtgatcgccgcagcgcagcgtgaaggtaaaacctgtgcgtttatcgatgctgaacacgcgctggacccaatctacgcacgtaaactgggcgtcgatatcgacaacctgctgtgctcccagccggacaccggcgagcaggcactggaaatctgtgacgccctggcgcgttctggcgcagtagacgttatcgtcgttgactccgtggcggcactgacgccgaaagcggaaatcgaaggcgaaatcggcgactctcacatgggccttgcggcacgtatgatgagccaggcgatgcgtaagctggcgggtaacctgaagcagtccaacacgctgctgatcttcatcaaccagatccgtatgaaaattggtgtgatgttcggtaacccggaaaccactaccggtggtaacgcgctgaaattctacgcctctgttcgtctcgacatccgtcgtatcggcgcggtgaaagagggcgaaaacgtggtgggtagcgaaacccgcgtgaaagtggtgaagaacaaaatcgctgcgccgtttaaacaggctgaattccagatcctctacggcgaaggtatcaacttctacggcgaactggttgacctgggcgtaaaagagaagctgatcgagaaagcaggcgcgtggtacagctacaaaggtgagaagatcggtcagggtaaagcgaatgcgactgcctggctgaaagataacccggaaaccgcgaaagagatcgagaagaaagtacgtgagttgctgctgagcaacccgaactcaacgccggatttctctgtagatgatagcgaaggcgtagcagaaactaacgaagatttttaa

SEQ ID NO: 44 - DNA, 1023 bp, synthetic construct
  source 1..1023: mol_type = other DNA
atctacagagaaatccggcgttgagttcgggttgctcagcagcaactcacgtactttcttctcgatctctttcgcggtttccgggttatctttcagccaggcagtcgcattcgctttaccctgaccgatcttctcacctttgtagctgtaccacgcgcctgctttctcgatcagcttctcttttacgcccaggtcaaccagttcgccgtagaagttgataccttcgccgtagaggatctggaattcagcctgtttaaacggcgcagcgattttgttcttcaccactttcacgcgggtttcgctacccaccacgttttcgccctctttcaccgcgccgatacgacggatgtcgagacgaacagaggcgtagaatttcagcgcgttaccaccggtagtggtttccgggttaccgaacatcacaccaattttcatacggatctggttgatgaagatcagcagcgtgttggactgcttcaggttacccgccagcttacgcatcgcctggctcatcatacgtgccgcaagacccatgtgagagtcgtcgatttcgccttcgatttccgctttcggcgtcagtgccgccacggagtcaacgacgataacgtctactgcgccagaacgcgccagggcgtcacagatttccagtgcctgctcgccggtgtccggctgggagcacagcaggttgtcgatatcgacgcccagtttacgtgcgtagattgggtccagcgcgtgttcagcatcgataaacgcacaggttttaccttcacgctgcgctgcggcgatcacctgcagcgtcagcgtggttttaccggaagattccggtccgtagatttcgacgatacggcccatcggcagaccacctgccccaagcgcgatatccagtgaaagcgaaccggtagagatggtttccacatccatggaacggtcttcacccaggcgcatgatggagcctttaccaaattgtttctcaatctggcccagtgctgccgccaacgctttctgtttgttttcgtcgatagccat

SEQ ID NO: 45 - DNA, 20 bp, unidentified
  source 1..20: mol_type = other DNA
atggggccacgatttccgcc

SEQ ID NO: 46 - DNA, 20 bp, synthetic construct
  source 1..20: mol_type = other DNA
gggctggcctgcttacgagg

SEQ ID NO: 47 - DNA, 20 bp, synthetic construct
  source 1..20: mol_type = other DNA
ggctcatcatacgtgccgca

SEQ ID NO: 48 - DNA, 1000 bp, synthetic construct
  source 1..1000: mol_type = other DNA
agttaggcttaagttacccgatcaccaaacatgtgcgcctttatactcaggtttacagcggctatggcgaatcgctcatcgactataacttcaaccagacccgtgtcggtgtgggggttatgctaaacgatttgttttgatgaacggttgagtggttggcaaatctggaatccagcatccaggattaccctctcagagactaaaagcattgcagtttctcgcgcaggcgctgaaaatagcgcctgtttttatttcaggcaatcggggtgaatgtggcgcaggcggaagtgttgaatctggagtccggagctaaacaggttttacaagaaacctttggctaccaacagtttcgccccggccaggaagaaattatcgacactgtgctttccggccgcgattgcctcgtcgtcatgcccactggtggcggaaaatccctttgctatcaaatccctgccttattgctaaacggccttaccgtggttgtttcaccgctgatttcgctgttcgccaaattacgcaaactgcgtaaatcgatagccgatgaaagtaatgtcccgccgtacgtggtgtttaacgacgcaaccttgattgagatggctgaacagatgccgatcaccgccagcgaaatgctcagcgttaacggcgttgggatgcgcaagctggaacgctttggcaaaccgtttatggcgctgattcgtgcgcatgttgatggcgatgacgaagagtagtcagcagcataaaaaagtgccagtatgaagactccgtaaacgtttcccccgcgagtcaaatgtatgttgatgttatttctcaccgtcgccatggtgcacattgtggcgcttatgagccccggtcccgatttcttttttgtctctcagaccgctgtcagtcgttcccgtaaagaagcgatgatgggcgtgctgggcattacctgcggcgtaatggtttgggctgggattgcgctgcttggcctgcatttgattatcgaaaaaatggcctggct

SEQ ID NO: 49 - DNA, 2417 bp, synthetic construct
  source 1..2417: mol_type = other DNA
tggttatcgatatcatgatactgcggcggggcgctaaaacgaagggaagaagcattagtgtaattaattaaagcaagataatacgtatgtttgatcaattttcgaggcgataaccggccataaaaaagcgcaacgtagaacaggaattattctcacgaaagaaatccattaccatctctttatccagtccatagcggcgcgtcagaatacccgcttcccaggcgctaagctggcgatctccggtcttttcgtacatccggtgtgagtagcctaatacaaaaccgcgtttataatcggcacagaattttgtcacattaaccgcactgtcggcatgcgttgcttttaatcccgccattaagcctttaccaaaatggttattcatcgttcacctcattcgctatatattgtcatatatagcgatattttaggcaaagaacgacttttgcgcacgctattttttcatgcttgtttaagacgtaatcccgtaagagataaacctattccgacaccatcgaatggtgcaaaacctttcgcggtatggcatgatagcgcccggaagagagtcaattcagggtggtgaatgtgaaaccagtaacgttatacgatgtcgcagagtatgccggtgtctcttatcagaccgtttcccgcgtggtgaaccaggccagccacgtttctgcgaaaacgcgggaaaaagtggaagcggcgatggcggagctgaattacattcccaaccgcgtggcacaacaactggcgggcaaacagtcgttgctgattggcgttgccacctccagtctggccctgcacgcgccgtcgcaaattgtcgcggcgattaaatctcgcgccgatcaactgggtgccagcgtggtggtgtcgatggtagaacgaagcggcgtcgaagcctgtaaagcggcggtgcacaatcttctcgcgcaacgcgtcagtgggctgatcattaactatccgctggatgaccaggatgccattgctgtggaagctgcctgcactaatgttccggcgttatttcttgatgtctctgaccagacacccatcaacagtattattttctcccatgaagacggtacgcgactgggcgtggagcatctggtcgcattgggtcaccagcaaatcgcgctgttagcgggcccattaagttctgtctcggcgcgtctgcgtctggctggctggcataaatatctcactcgcaatcaaattcagccgatagcggaacgggaaggcgactggagtgccatgtccggttttcaacaaaccatgcaaatgctgaatgagggcatcgttcccactgcgatgctggttgccaacgatcagatggcgctgggcgcaatgcgcgccattaccgagtccgggctgcgcgttggtgcggatatctcggtagtgggatacgacgataccgaagacagctcatgttatatcccgccgttaaccaccatcaaacaggattttcgcctgctggggcaaaccagcgtggaccgcttgctgcaactctctcagggccaggcggtgaagggcaatcagctgttgcccgtctcactggtgaaaagaaaaaccaccctggcgcccaatacgcaaaccgcctctccccgcgcgttggccgattcattaatgcagctggcacgacaggtttcccgactggaaagcgggcagtgaaattcgcgcaacgcaattaatgtaagttagctcactcattaggcaccaaataaaacgaaaggctcagtcgaaagactgggcctttcgttttatctgttgtttgtcggtgaacgctctcctgagtaggacaaatccgccgggagcggatttgaacgttgcgaagcaacggcccggagggtggcgggcaggacgcccgccataaactgccaggcatcaaattaagcagaaggccatcctgacggatggccttttagtaatccagcaactcttgtgggaaatctttggcggttaaacgcggcatcgttgcactcctcagttggtgtttttttaagcaaagcataagcacgtatttttgcccagtttttcgtcactctgtgagccagactacgggatacgcgctggcgaatcgctaaactagaaacattgtttcgaaattgaacggtggaaaggagaggtcatggtctggttagcgaatcccgaacgttacgggcagatgcaataccgctattgcggaaaaagtggtttacgcctgcccgcgttatcgctcggtttatggcacaatttcggtcacgttaacgcgctggaatcacagcgtgcgatcctgcgtaaagcgtttgatttgggcattacgcactttgatttagccaacaattacgggccgcctccaggaagcgcagaagagaactttggtcgcctgctgcgggaggattttgccgcttatcgcgatgaactgattatctctaccaaggctg

SEQ ID NO: 50 - DNA, 1080 bp, synthetic construct
  source 1..1080: mol_type = other DNA
atctacagagaaatccggcgttgagttcgggttgctcagcagcaactcacgtactttcttctcgatctctttcgcggtttccgggttatctttcagccaggcagtcgcattcgctttaccctgaccgatcttctcacctttgtagctgtaccacgcgcctgctttctcgatcagcttctcttttacgcccaggtcaaccagttcgccgtagaagttgataccttcgccgtagaggatctggaattcagcctgtttaaacggcgcagcgattttgttcttcaccactttcacgcgggtttcgctacccaccacgttttcgccctctttcaccgcgccgatacgacggatgtcgagacgaacagaggcgtagaatttcagcgcgttaccaccggtagtggtttccgggttaccgaacatcacaccaattttcatacggatctggttgatgaagatcagcagcgtgttggactgcttcaggttacccgccagcttacgcatcgcctggctcatcatacgtgccgcaagacccatgtgagagtcgtcgatttcgccttcgatttccgctttcggcgtcagtgccgccacggagtcaacgacgataacgtctactgcgccagaacgcgccagggcgtcacagatttccagtgcctgctcgccggtgtccggctgggagcacagcaggttgtcgatatcgacgcccagtttacgtgcgtagattgggtccagcgcgtgttcagcatcgataaacgcacaggttttaccttcacgctgcgctgcggcgatcacctgcagcgtcagcgtggttttaccggaagattccggtccgtagatttcgacgatacggcccatcggcagaccacctgccccaagcgcgatatccagtgaaagcgaaccggtagagatggtttccacatccatggaacggtcttcacccaggcgcatgatggagcctttaccaaattgtttctcaatctggcccagtgctgccgccaacgctttctgtttgttttcgtcgatagccatttttactcctgtcatgccgggtaataccggatagtcaatatgttctgttgaagcaat